European Patent Application EP 4 434 543 A2, published September 25, 2024. Title: Polypeptide Variants and Uses Thereof. Applicant: Genmab B.V. Application EP PCT/EP2013/050429, filed January 10, 2013. The sequence listing filed with the application follows.

SEQUENCE LISTING (18 sequences)

SEQ ID NO: 1 - protein, 330 aa, Homo sapiens
ASTKGPSVFPLAPSSKSTSGGTAALGCLVKDYFPEPVTVSWNSGALTSGVHTFPAVLQSSGLYSLSSVVTVPSSSLGTQTYICNVNHKPSNTKVDKKVEPKSCDKTHTCPPCPAPELLGGPSVFLFPPKPKDTLMISRTPEVTCVVVDVSHEDPEVKFNWYVDGVEVHNAKTKPREEQYNSTYRVVSVLTVLHQDWLNGKEYKCKVSNKALPAPIEKTISKAKGQPREPQVYTLPPSRDEMTKNQVSLTCLVKGFYPSDIAVEWESNGQPENNYKTTPPVLDSDGSFFLYSKLTVDKSRWQQGNVFSCSVMHEALHNHYTQKSLSLSPGK

SEQ ID NO: 2 - protein, 326 aa, Homo sapiens
ASTKGPSVFPLAPCSRSTSESTAALGCLVKDYFPEPVTVSWNSGALTSGVHTFPAVLQSSGLYSLSSVVTVPSSNFGTQTYTCNVDHKPSNTKVDKTVERKCCVECPPCPAPPVAGPSVFLFPPKPKDTLMISRTPEVTCVVVDVSHEDPEVQFNWYVDGVEVHNAKTKPREEQFNSTFRVVSVLTVVHQDWLNGKEYKCKVSNKGLPAPIEKTISKTKGQPREPQVYTLPPSREEMTKNQVSLTCLVKGFYPSDIAVEWESNGQPENNYKTTPPMLDSDGSFFLYSKLTVDKSRWQQGNVFSCSVMHEALHNHYTQKSLSLSPGK

SEQ ID NO: 3 - protein, 377 aa, Homo sapiens
ASTKGPSVFPLAPCSRSTSGGTAALGCLVKDYFPEPVTVSWNSGALTSGVHTFPAVLQSSGLYSLSSVVTVPSSSLGTQTYTCNVNHKPSNTKVDKRVELKTPLGDTTHTCPRCPEPKSCDTPPPCPRCPEPKSCDTPPPCPRCPEPKSCDTPPPCPRCPAPELLGGPSVFLFPPKPKDTLMISRTPEVTCVVVDVSHEDPEVQFKWYVDGVEVHNAKTKPREEQYNSTFRVVSVLTVLHQDWLNGKEYKCKVSNKALPAPIEKTISKTKGQPREPQVYTLPPSREEMTKNQVSLTCLVKGFYPSDIAVEWESSGQPENNYNTTPPMLDSDGSFFLYSKLTVDKSRWQQGNIFSCSVMHEALHNRFTQKSLSLSPGK

SEQ ID NO: 4 - protein, 327 aa, Homo sapiens
ASTKGPSVFPLAPCSRSTSESTAALGCLVKDYFPEPVTVSWNSGALTSGVHTFPAVLQSSGLYSLSSVVTVPSSSLGTKTYTCNVDHKPSNTKVDKRVESKYGPPCPSCPAPEFLGGPSVFLFPPKPKDTLMISRTPEVTCVVVDVSQEDPEVQFNWYVDGVEVHNAKTKPREEQFNSTYRVVSVLTVLHQDWLNGKEYKCKVSNKGLPSSIEKTISKAKGQPREPQVYTLPPSQEEMTKNQVSLTCLVKGFYPSDIAVEWESNGQPENNYKTTPPVLDSDGSFFLYSRLTVDKSRWQEGNVFSCSVMHEALHNHYTQKSLSLSLGK

SEQ ID NO: 5 - protein, 330 aa, Homo sapiens
ASTKGPSVFPLAPSSKSTSGGTAALGCLVKDYFPEPVTVSWNSGALTSGVHTFPAVLQSSGLYSLSSVVTVPSSSLGTQTYICNVNHKPSNTKVDKRVEPKSCDKTHTCPPCPAPELLGGPSVFLFPPKPKDTLMISRTPEVTCVVVDVSHEDPEVKFNWYVDGVEVHNAKTKPREEQYNSTYRVVSVLTVLHQDWLNGKEYKCKVSNKALPAPIEKTISKAKGQPREPQVYTLPPSREEMTKNQVSLTCLVKGFYPSDIAVEWESNGQPENNYKTTPPVLDSDGSFFLYSKLTVDKSRWQQGNVFSCSVMHEALHNHYTQKSLSLSPGK

SEQ ID NO: 6 - protein, 201 aa, Homo sapiens
PKDTLMISRTPEVTCVVVDVSHEDPEVKFNWYVDGVEVHNAKTKPREEQYNSTYRVVSVLTVLHQDWLNGKEYKCKVSNKALPAPIEKTISKAKGQPREPQVYTLPPSRDELTKNQVSLTCLVKGFYPSDIAVEWESNGQPENNYKTTPPVLDSDGSFFLYSKLTVDKSRWQQGNVFSCSVMHEALHNHYTQKSLSLSPGK

SEQ ID NO: 7 - protein, 201 aa, Homo sapiens
PKDTLMISRTPEVTCVVVDVSHEDPEVKFNWYVDGVEVHNAKTKPREEQYNSTYRVVSVLTVLHQDWLNGKEYKCKVSNKALPAPIEKTISKAKGQPREPQVYTLPPSREEMTKNQVSLTCLVKGFYPSDIAVEWESNGQPENNYKTTPPVLDSDGSFFLYSKLTVDKSRWQQGNVFSCSVMHEALHNHYTQKSLSLSPGK

SEQ ID NO: 8 - protein, 201 aa, Homo sapiens
PKDTLMISRTPEVTCVVVDVSHEDPEVQFNWYVDGVEVHNAKTKPREEQFNSTFRVVSVLTVVHQDWLNGKEYKCKVSNKGLPAPIEKTISKTKGQPREPQVYTLPPSREEMTKNQVSLTCLVKGFYPSDIAVEWESNGQPENNYKTTPPMLDSDGSFFLYSKLTVDKSRWQQGNVFSCSVMHEALHNHYTQKSLSLSPGK

SEQ ID NO: 9 - protein, 201 aa, Homo sapiens
PKDTLMISRTPEVTCVVVDVSHEDPEVQFKWYVDGVEVHNAKTKPREEQYNSTFRVVSVLTVLHQDWLNGKEYKCKVSNKALPAPIEKTISKTKGQPREPQVYTLPPSREEMTKNQVSLTCLVKGFYPSDIAVEWESSGQPENNYNTTPPMLDSDGSFFLYSKLTVDKSRWQQGNIFSCSVMHEALHNRFTQKSLSLSPGK

SEQ ID NO: 10 - protein, 201 aa, Homo sapiens
PKDTLMISRTPEVTCVVVDVSQEDPEVQFNWYVDGVEVHNAKTKPREEQFNSTYRVVSVLTVLHQDWLNGKEYKCKVSNKGLPSSIEKTISKAKGQPREPQVYTLPPSQEEMTKNQVSLTCLVKGFYPSDIAVEWESNGQPENNYKTTPPVLDSDGSFFLYSRLTVDKSRWQEGNVFSCSVMHEALHNHYTQKSLSLSLGK

SEQ ID NO: 11 - protein, 204 aa, Homo sapiens
SPFDLFIRKSPTITCLVVDLAPSKGTVNLTWSRASGKPVNHSTRKEEKQRNGTLTVTSTLPVGTRDWIEGETYQCRVTHPHLPRALMRSTTKTSGPRAAPEVYAFATPEWPGSRDKRTLACLIQNFMPEDISVQWLHNEVQLPDARHSTTQPRKTKGSGFFVFSRLEVTRAEWEQKDEFICRAVHEAASPSQTVQRAVSVNPGK

SEQ ID NO: 12 - protein, 221 aa, Homo sapiens
ALEDLLLGSEANLTCTLTGLRDASGVTFTWTPSSGKSAVQGPPERDLCGCYSVSSVLPGCAEPWNHGKTFTCTAAYPESKTPLTATLSKSGNTFRPEVHLLPPPSEELALNELVTLTCLARGFSPKDVLVRWLQGSQELPREKYLTWASRQEPSQGTTTFAVTSILRVAAEDWKKGDTFSCMVGHEALPLAFTQKTIDRLAGKPTHVNVSVVMAEVDGTCY

SEQ ID NO: 13 - protein, 221 aa, Homo sapiens
ALEDLLLGSEANLTCTLTGLRDASGATFTWTPSSGKSAVQGPPERDLCGCYSVSSVLPGCAQPWNHGETFTCTAAHPELKTPLTANITKSGNTFRPEVHLLPPPSEELALNELVTLTCLARGFSPKDVLVRWLQGSQELPREKYLTWASRQEPSQGTTTFAVTSILRVAAEDWKKGDTFSCMVGHEALPLAFTQKTIDRLAGKPTHVNVSVVMAEVDGTCY

SEQ ID NO: 14 - protein, 223 aa, Homo sapiens
SFASIFLTKSTKLTCLVTDLTTYDSVTISWTRQNGEAVKTHTNISESHPNATFSAVGEASICEDDWNSGERFTCTVTHTDLPSPLKQTISRPKGVALHRPDVYLLPPAREQLNLRESATITCLVTGFSPADVFVQWMQRGQPLSPEKYVTSAPMPEPQAPGRYFAHSILTVSEEEWNTGETYTCVAHEALPNRVTERTVDKSTGKPTLYNVSLVMSDTAGTCY

SEQ ID NO: 15 - protein, 209 aa, Homo sapiens
AVQDLWLRDKATFTCFVVGSDLKDAHLTWEVAGKVPTGGVEEGLLERHSNGSQSQHSRLTLPRSLWNAGTSVTCTLNHPSLPPQRLMALREPAAQAPVKLSLNLLASSDPPEAASWLLCEVSGFSPPNILLMWLEDQREVNTSGFAPARPPPQPGSTTFWAWSVLRVPAPPSPQPATYTCVVSHEDSRTLLNASRSLEVSYVTDHGPMK

SEQ ID NO: 16 - protein, 454 aa, Homo sapiens
VQLVESGGGVVQPGRSLRLSCAASGFTFSTYGMHWVRQAPGKGLEWVAVIWDDGSYKYYGDSVKGRFTISRDNSKNTLYLQMNSLRAEDTAVYYCARDGITMVRGVMKDYFDYWGQGTLVTVSSASTKGPSVFPLAPSSKSTSGGTAALGCLVKDYFPEPVTVSWNSGALTSGVHTFPAVLQSSGLYSLSSVVTVPSSSLGTQTYICNVNHKPSNTKVDKRVEPKSCDKTHTCPPCPAPELLGGPSVFLFPPKPKDTLMISRTPEVTCVVVDVSHEDPEVKFNWYVDGVEVHNAKTKPREEQYNSTYRVVSVLTVLHQDWLNGKEYKCKVSNKALPAPIEKTISKAKGQPREPQVYTLPPSRDELTKNQVSLTCLVKGFYPSDIAVEWESNGQPENNYKTTPPVLDSDGSFFLYSKLTVDKSRWQQGNVFSCSVMHEALHNHYTQKSLSLSPGK

SEQ ID NO: 17 - protein, 451 aa, Homo sapiens
VQLVESGGGVVQPGRSLRLSCAASGFTFSTYGMHWVRQAPGKGLEWVAVIWDDGSYKYYGDSVKGRFTISRDNSKNTLYLQMNSLRAEDTAVYYCARDGITMVRGVMKDYFDYWGQGTLVTVSSASTKGPSVFPLAPCSRSTSEGTAALGCLVKDYFPEPVTVSWNSGALTSGVHTFPAVLQSSGLYSLSSVVTVPSSSLGTKTYTCNVNHKPSNTKVDKRVESKYGPPCPSCPAPEFLGGPSVFLFPPKPKDTLMISRTPEVTCVVVDVSQEDPEVQFNWYVDGVEVHNAKTKPREEQFNSTYRVVSVLTVLHQDWLNGKEYKCKVSNKGLPSSIEKTISKAKGQPREPQVYTLPPSQEEMTKNQVSLTCLVKGFYPSDIAVEWESNGQPENNYKTTPPVLDSDGSFFLYSRLTVDKSRWQEGNVFSCSVMHEALHNHYTQKSLSLSLGK

SEQ ID NO: 18 - protein, 97 aa, Homo sapiens
NVNHKPSNTKVDKRVELKTPLGDTTHTCPRCPEPKSCDTPPPCPRCPEPKSCDTPPPCPRCPEPKSCDTPPPCPRCPAPELLGGPSVFLFPPKPKDT